European Patent Application EP 4 144 359 A1, published March 8, 2023. Title: Peptides having an activity of mobilizing mesenchymal stem cells. Applicant: StemRIM Inc. Osaka University. The sequence listing filed with the application follows.

SEQUENCE LISTING (22 sequences)

SEQ ID NO: 1 - protein, 30 aa, Artificial Sequence
  An artificially synthesized peptide sequence
IMWLCQYFFQCHKCAVKKKTWKEKKDRRHP

SEQ ID NO: 2 - protein, 27 aa, Artificial Sequence
  An artificially synthesized peptide sequence
IMWLCQYFFQCHKCAVKKKTWKEKKDR

SEQ ID NO: 3 - protein, 26 aa, Artificial Sequence
  An artificially synthesized peptide sequence
IMWLCQYFFQCHKCAVKKKTWKEKKD

SEQ ID NO: 4 - protein, 25 aa, Artificial Sequence
  An artificially synthesized peptide sequence
IMWLCQYFFQCHKCAVKKKTWKEKK

SEQ ID NO: 5 - protein, 24 aa, Artificial Sequence
  An artificially synthesized peptide sequence
IMWLCQYFFQCHKCAVKKKTWKEK

SEQ ID NO: 6 - protein, 23 aa, Artificial Sequence
  An artificially synthesized peptide sequence
IMWLCQYFFQCHKCAVKKKTWKE

SEQ ID NO: 7 - protein, 19 aa, Artificial Sequence
  An artificially synthesized peptide sequence
IMWLCQYFFQCHKCAVKKK

SEQ ID NO: 8 - protein, 18 aa, Artificial Sequence
  An artificially synthesized peptide sequence
IMWLCQYFFQCHKCAVKK

SEQ ID NO: 9 - protein, 16 aa, Artificial Sequence
  An artificially synthesized peptide sequence
IMWLCQYFFQCHKCAV

SEQ ID NO: 10 - protein, 15 aa, Artificial Sequence
  An artificially synthesized peptide sequence
IMWLCQYFFQCHKCA

SEQ ID NO: 11 - protein, 25 aa, Artificial Sequence
  An artificially synthesized peptide sequence
QYFFQCHKCAVKKKTWKEKKDRRHP

SEQ ID NO: 12 - protein, 20 aa, Artificial Sequence
  An artificially synthesized peptide sequence
CHKCAVKKKTWKEKKDRRHP

SEQ ID NO: 13 - protein, 19 aa, Artificial Sequence
  An artificially synthesized peptide sequence
HKCAVKKKTWKEKKDRRHP

SEQ ID NO: 14 - protein, 18 aa, Artificial Sequence
  An artificially synthesized peptide sequence
KCAVKKKTWKEKKDRRHP

SEQ ID NO: 15 - protein, 15 aa, Artificial Sequence
  An artificially synthesized peptide sequence
VKKKTWKEKKDRRHP

SEQ ID NO: 16 - protein, 14 aa, Artificial Sequence
  An artificially synthesized peptide sequence
KKKTWKEKKDRRHP

SEQ ID NO: 17 - protein, 13 aa, Artificial Sequence
  An artificially synthesized peptide sequence
KKTWKEKKDRRHP

SEQ ID NO: 18 - protein, 12 aa, Artificial Sequence
  An artificially synthesized peptide sequence
KTWKEKKDRRHP

SEQ ID NO: 19 - protein, 11 aa, Artificial Sequence
  An artificially synthesized peptide sequence
QYFFQCHKCAV

SEQ ID NO: 20 - DNA, 90 bp, Artificial Sequence
  An artificially synthesized nucleotide sequence
atcatgtggctgtgccagtacttcttccagtgccacaagtgcgccgtgaagaagaagacctggaaggagaagaaggacaggaggcacccc

SEQ ID NO: 21 - DNA, 39 bp, Artificial Sequence
  An artificially synthesized nucleotide sequence
aagaagacctggaaggagaagaaggacagaagacacccc

SEQ ID NO: 22 - DNA, 33 bp, Artificial Sequence
  An artificially synthesized nucleotide sequence
cagtacttcttccagtgccacaagtgcgccgtg